European Patent Specification EP 4 127 220 B1, published June 5, 2024. Title: METHOD AND COMPOSITIONS FOR PREPARING NORMALIZED NUCLEIC ACID LIBRARIES. Applicant: Christiansen, Lena Pokholok, Dmitry Steemers, Frank J. Pantoja, Rigo Chu, Megan Iavicoli, Patrizia Chang, Weihua Brodin, Jeffrey Vermaas, Eric Thomas, Jerushah Zhang, Fan. The sequence listing filed with the application follows.

SEQUENCE LISTING (9 sequences)

SEQ ID NO: 1 - DNA, 20 bp, Artificial Sequence
  Primer P5
aatgatacggcgaccaccga

SEQ ID NO: 2 - DNA, 24 bp, Artificial Sequence
  Primer P7
caagcagaagacggcatacgagat

SEQ ID NO: 3 - DNA, 26 bp, Artificial Sequence
  GGA-primer
aaaaaggaggaggaggaggaggaaaa

SEQ ID NO: 4 - DNA, 30 bp, Artificial Sequence
  AAG-primer
aagaagaagaagaagaagaagaagaagaaa

SEQ ID NO: 5 - DNA, 26 bp, Artificial Sequence
  GGA-amplification
aaaaaggaggaggaggaggaggaaaa

SEQ ID NO: 6 - DNA, 37 bp, Artificial Sequence
  AAGGGGT-primer
gggaagaagtaagaagaatgaagtaagaagatagaaa

SEQ ID NO: 7 - DNA, 50 bp, Artificial Sequence
  P5-GGA
aatgatacggcgaccaccgagatctacacggaggaggaggaggaggaaaa

SEQ ID NO: 8 - DNA, 61 bp, Artificial Sequence
  AAGGGGT-P7
caagcagaagacggcatacgagatgggaagaagtaagaagaatgaagtaagaagatagaaa

SEQ ID NO: 9 - DNA, 24 bp, Artificial Sequence
  CS Index 1 primer
ctccacactacctcaaccatcact